European Patent Specification EP 3 398 968 B1, published June 12, 2024. Title: PCSK9 ANTIBODY, ANTIGEN-BINDING FRAGMENTS THEREOF AND MEDICAL APPLICATION THEREOF. Applicant: JIANGSU HENGRUI MEDICINE CO.,LTD  SHANGHAI HENGRUI PHARMACEUTICAL CO.,LTD. The sequence listing filed with the application follows.

SEQUENCE LISTING (33 sequences)

SEQ ID NO: 1 - protein, 698 aa, Artificial
  PCSK9 with his tag:PCSK9-His6, used as immunogen for immunizing mice or as a detection reagent
MGTVSSRRSWWPLPLLLLLLLLLGPAGARAQEDEDGDYEELVLALRSEEDGLAEAPEHGTTATFHRCAKDPWRLPGTYVVVLKEETHLSQSERTARRLQAQAARRGYLTKILHVFHGLLPGFLVKMSGDLLELALKLPHVDYIEEDSSVFAQSIPWNLERITPPRYRADEYQPPDGGSLVEVYLLDTSIQSDHREIEGRVMVTDFENVPEEDGTRFHRQASKCDSHGTHLAGVVSGRDAGVAKGASMRSLRVLNCQGKGTVSGTLIGLEFIRKSQLVQPVGPLVVLLPLAGGYSRVLNAACQRLARAGVVLVTAAGNFRDDACLYSPASAPEVITVGATNAQDQPVTLGTLGTNFGRCVDLFAPGEDIIGASSDCSTCFVSQSGTSQAAAHVAGIAAMMLSAEPELTLAELRQRLIHFSAKDVINEAWFPEDQRVLTPNLVAALPPSTHGAGWQLFCRTVWSAHSGPTRMATAVARCAPDEELLSCSSFSRSGKRRGERMEAQGGKLVCRAHNAFGGEGVYAIARCCLLPQANCSVHTAPPAEASMGTRVHCHQQGHVLTGCSSHWEVEDLGTHKPPVLRPRGQPNQCVGHREASIHASCCHAPGLECKVKEHGIPAPQEQVTVACEEGWTLTGCSALPGTSHVLGAYAVDNTCVVRSRDVSTTGSTSEGAVTAVAICCRSRHLAQASQELQHHHHHH

SEQ ID NO: 2 - protein, 714 aa, ARTIFICIAL
  PCSK9 with PADRE peptide and His tag: PCSK9-PADRE-His6, as an immunogen, contained PADRE peptide can promote immunization
MGTVSSRRSWWPLPLLLLLLLLLGPAGARAQEDEDGDYEELVLALRSEEDGLAEAPEHGTTATFHRCAKDPWRLPGTYVVVLKEETHLSQSERTARRLQAQAARRGYLTKILHVFHGLLPGFLVKMSGDLLELALKLPHVDYIEEDSSVFAQSIPWNLERITPPRYRADEYQPPDGGSLVEVYLLDTSIQSDHREIEGRVMVTDFENVPEEDGTRFHRQASKCDSHGTHLAGVVSGRDAGVAKGASMRSLRVLNCQGKGTVSGTLIGLEFIRKSQLVQPVGPLVVLLPLAGGYSRVLNAACQRLARAGVVLVTAAGNFRDDACLYSPASAPEVITVGATNAQDQPVTLGTLGTNFGRCVDLFAPGEDIIGASSDCSTCFVSQSGTSQAAAHVAGIAAMMLSAEPELTLAELRQRLIHFSAKDVINEAWFPEDQRVLTPNLVAALPPSTHGAGWQLFCRTVWSAHSGPTRMATAVARCAPDEELLSCSSFSRSGKRRGERMEAQGGKLVCRAHNAFGGEGVYAIARCCLLPQANCSVHTAPPAEASMGTRVHCHQQGHVLTGCSSHWEVEDLGTHKPPVLRPRGQPNQCVGHREASIHASCCHAPGLECKVKEHGIPAPQEQVTVACEEGWTLTGCSALPGTSHVLGAYAVDNTCVVRSRDVSTTGSTSEGAVTAVAICCRSRHLAQASQELQGSGAKFVAAWTLKAAAHHHHHH

SEQ ID NO: 3 - protein, 704 aa, ARTIFICIAL
  Fusion protein of PCSK9 containing TEV cleavage site and His tag: PCSK9-TEV-His6, N-PCSK9 (N terminal pCSK9 domain) as an immunogen can be obtained via TEV enzyme digestion
MGTVSSRRSWWPLPLLLLLLLLLGPAGARAQEDEDGDYEELVLALRSEEDGLAEAPEHGTTATFHRCAKDPWRLPGTYVVVLKEETHLSQSERTARRLQAQAARRGYLTKILHVFHGLLPGFLVKMSGDLLELALKLPHVDYIEEDSSVFAQSIPWNLERITPPRYRADEYQPPDGGSLVEVYLLDTSIQSDHREIEGRVMVTDFENVPEEDGTRFHRQASKCDSHGTHLAGVVSGRDAGVAKGASMRSLRVLNCQGKGTVSGTLIGLEFIRKSQLVQPVGPLVVLLPLAGGYSRVLNAACQRLARAGVVLVTAAGNFRDDACLYSPASAPEVITVGATNAQDQPVTLGTLGTNFGRCVDLFAPGEDIIGASSDCSTCFVSQSGTSQAAAHVAGIAAMMLSAEPELTLAELRQRLIHFSAKDVINEAWFPEDQRVLTPNLVAALPPSTHENLYFQGAGWQLFCRTVWSAHSGPTRMATAVARCAPDEELLSCSSFSRSGKRRGERMEAQGGKLVCRAHNAFGGEGVYAIARCCLLPQANCSVHTAPPAEASMGTRVHCHQQGHVLTGCSSHWEVEDLGTHKPPVLRPRGQPNQCVGHREASIHASCCHAPGLECKVKEHGIPAPQEQVTVACEEGWTLTGCSALPGTSHVLGAYAVDNTCVVRSRDVSTTGSTSEGAVTAVAICCRSRHLAQASQELQHHHHHH

SEQ ID NO: 4 - protein, 698 aa, ARTIFICIAL
  PCSK9-D374Y mutant protein with His tag: PCSK9-D374Y-His6, as a detection reagent
MGTVSSRRSWWPLPLLLLLLLLLGPAGARAQEDEDGDYEELVLALRSEEDGLAEAPEHGTTATFHRCAKDPWRLPGTYVVVLKEETHLSQSERTARRLQAQAARRGYLTKILHVFHGLLPGFLVKMSGDLLELALKLPHVDYIEEDSSVFAQSIPWNLERITPPRYRADEYQPPDGGSLVEVYLLDTSIQSDHREIEGRVMVTDFENVPEEDGTRFHRQASKCDSHGTHLAGVVSGRDAGVAKGASMRSLRVLNCQGKGTVSGTLIGLEFIRKSQLVQPVGPLVVLLPLAGGYSRVLNAACQRLARAGVVLVTAAGNFRDDACLYSPASAPEVITVGATNAQDQPVTLGTLGTNFGRCVDLFAPGEDIIGASSYCSTCFVSQSGTSQAAAHVAGIAAMMLSAEPELTLAELRQRLIHFSAKDVINEAWFPEDQRVLTPNLVAALPPSTHGAGWQLFCRTVWSAHSGPTRMATAVARCAPDEELLSCSSFSRSGKRRGERMEAQGGKLVCRAHNAFGGEGVYAIARCCLLPQANCSVHTAPPAEASMGTRVHCHQQGHVLTGCSSHWEVEDLGTHKPPVLRPRGQPNQCVGHREASIHASCCHAPGLECKVKEHGIPAPQEQVTVACEEGWTLTGCSALPGTSHVLGAYAVDNTCVVRSRDVSTTGSTSEGAVTAVAICCRSRHLAQASQELQHHHHHH

SEQ ID NO: 5 - protein, 719 aa, ARTIFICIAL
  PCSK9 protein inserted with biotin receiving peptide BP15 and His tag: PCSK9-BP15-His6. As a detection reagent, biotin will be labeled to BP15 peptide position during expression, avoiding the biotin labeling in vitro and consequently avoiding possible conformational changes.
MGTVSSRRSWWPLPLLLLLLLLLGPAGARAQEDEDGDYEELVLALRSEEDGLAEAPEHGTTATFHRCAKDPWRLPGTYVVVLKEETHLSQSERTARRLQAQAARRGYLTKILHVFHGLLPGFLVKMSGDLLELALKLPHVDYIEEDSSVFAQSIPWNLERITPPRYRADEYQPPDGGSLVEVYLLDTSIQSDHREIEGRVMVTDFENVPEEDGTRFHRQASKCDSHGTHLAGVVSGRDAGVAKGASMRSLRVLNCQGKGTVSGTLIGLEFIRKSQLVQPVGPLVVLLPLAGGYSRVLNAACQRLARAGVVLVTAAGNFRDDACLYSPASAPEVITVGATNAQDQPVTLGTLGTNFGRCVDLFAPGEDIIGASSDCSTCFVSQSGTSQAAAHVAGIAAMMLSAEPELTLAELRQRLIHFSAKDVINEAWFPEDQRVLTPNLVAALPPSTHGAGWQLFCRTVWSAHSGPTRMATAVARCAPDEELLSCSSFSRSGKRRGERMEAQGGKLVCRAHNAFGGEGVYAIARCCLLPQANCSVHTAPPAEASMGTRVHCHQQGHVLTGCSSHWEVEDLGTHKPPVLRPRGQPNQCVGHREASIHASCCHAPGLECKVKEHGIPAPQEQVTVACEEGWTLTGCSALPGTSHVLGAYAVDNTCVVRSRDVSTTGSTSEGAVTAVAICCRSRHLAQASQELQGSTSGSGLNDIFEAQKIEWHEHHHHHH

SEQ ID NO: 6 - protein, 719 aa, ARTIFICIAL
  PCSK9 D374Y mutant protein inserted with biotin receiving peptide BP15 and His tag: PCSK9-D374Y-BP15-His6, as a detection protein
MGTVSSRRSWWPLPLLLLLLLLLGPAGARAQEDEDGDYEELVLALRSEEDGLAEAPEHGTTATFHRCAKDPWRLPGTYVVVLKEETHLSQSERTARRLQAQAARRGYLTKILHVFHGLLPGFLVKMSGDLLELALKLPHVDYIEEDSSVFAQSIPWNLERITPPRYRADEYQPPDGGSLVEVYLLDTSIQSDHREIEGRVMVTDFENVPEEDGTRFHRQASKCDSHGTHLAGVVSGRDAGVAKGASMRSLRVLNCQGKGTVSGTLIGLEFIRKSQLVQPVGPLVVLLPLAGGYSRVLNAACQRLARAGVVLVTAAGNFRDDACLYSPASAPEVITVGATNAQDQPVTLGTLGTNFGRCVDLFAPGEDIIGASSYCSTCFVSQSGTSQAAAHVAGIAAMMLSAEPELTLAELRQRLIHFSAKDVINEAWFPEDQRVLTPNLVAALPPSTHGAGWQLFCRTVWSAHSGPTRMATAVARCAPDEELLSCSSFSRSGKRRGERMEAQGGKLVCRAHNAFGGEGVYAIARCCLLPQANCSVHTAPPAEASMGTRVHCHQQGHVLTGCSSHWEVEDLGTHKPPVLRPRGQPNQCVGHREASIHASCCHAPGLECKVKEHGIPAPQEQVTVACEEGWTLTGCSALPGTSHVLGAYAVDNTCVVRSRDVSTTGSTSEGAVTAVAICCRSRHLAQASQELQGSTSGSGLNDIFEAQKIEWHEHHHHHH

SEQ ID NO: 7 - protein, 802 aa, ARTIFICIAL
  PCSK9 receptor protein LDLR extracellular domain with Flag tag and His tag: LDLR-ECD-Flag-His6 as a detection reagent
MGPWGWKLRWTVALLLAAAGTAVGDRCERNEFQCQDGKCISYKWVCDGSAECQDGSDESQETCLSVTCKSGDFSCGGRVNRCIPQFWRCDGQVDCDNGSDEQGCPPKTCSQDEFRCHDGKCISRQFVCDSDRDCLDGSDEASCPVLTCGPASFQCNSSTCIPQLWACDNDPDCEDGSDEWPQRCRGLYVFQGDSSPCSAFEFHCLSGECIHSSWRCDGGPDCKDKSDEENCAVATCRPDEFQCSDGNCIHGSRQCDREYDCKDMSDEVGCVNVTLCEGPNKFKCHSGECITLDKVCNMARDCRDWSDEPIKECGTNECLDNNGGCSHVCNDLKIGYECLCPDGFQLVAQRRCEDIDECQDPDTCSQLCVNLEGGYKCQCEEGFQLDPHTKACKAVGSIAYLFFTNRHEVRKMTLDRSEYTSLIPNLRNVVALDTEVASNRIYWSDLSQRMICSTQLDRAHGVSSYDTVISRDIQAPDGLAVDWIHSNIYWTDSVLGTVSVADTKGVKRKTLFRENGSKPRAIVVDPVHGFMYWTDWGTPAKIKKGGLNGVDIYSLVTENIQWPNGITLDLLSGRLYWVDSKLHSISSIDVNGGNRKTILEDEKRLAHPFSLAVFEDKVFWTDIINEAIFSANRLTGSDVNLLAENLLSPEDMVLFHNLTQPRGVNWCERTTLSNGGCQYLCLPAPQINPHSPKFTCACPDGMLLARDMRSCLTEAEAAVATQETSTVRLKVSSTAVRTQHTTTRPVPDTSRLPGATPGLTTVEIVTMSHQALGDVAGRGNEKKPSSVRDYKDDDDKHHHHHH

SEQ ID NO: 8 - protein, 331 aa, ARTIFICIAL
  Fusion protein of abbreviated LDLR extracellular domain and hIgG1 Fc (with PCSK9 binding activity): LDLR-sECD-Fc (hIgG1) as a detection reagent
MEFGLSWLFLVAILKGVQCGTNECLDNNGGCSHVCNDLKIGYECLCPDGFQLVAQRRCEDIDECQDPDTCSQLCVNLEGGYKCQCEEGFQLDPHTKACKEPKSSDKTHTCPPCPAPELLGGPSVFLFPPKPKDTLMISRTPEVTCVVVDVSHEDPEVKFNWYVDGVEVHNAKTKPREEQYNSTYRVVSVLTVLHQDWLNGKEYKCKVSNKALPAPIEKTISKAKGQPREPQVYTLPPSRDELTKNQVSLTCLVKGFYPSDIAVEWESNGQPENNYKTTPPVLDSDGSFFLYSKLTVDKSRWQQGNVFSCSVMHEALHNHYTQKSLSLSPGK

SEQ ID NO: 9 - protein, 294 aa, ARTIFICIAL
  Fusion protein of more truncated LDLR extracellular domain and hIgG1 Fc (with PCSK9 binding activity): LDLR-ssECD-Fc (hIgG1) as a detection reagent
MEFGLSWLFLVAILKGVQCGTNECLDNNGGCSHVCNDLKIGYECLCPDGFQLVAQRRCEDIDEPKSSDKTHTCPPCPAPELLGGPSVFLFPPKPKDTLMISRTPEVTCVVVDVSHEDPEVKFNWYVDGVEVHNAKTKPREEQYNSTYRVVSVLTVLHQDWLNGKEYKCKVSNKALPAPIEKTISKAKGQPREPQVYTLPPSRDELTKNQVSLTCLVKGFYPSDIAVEWESNGQPENNYKTTPPVLDSDGSFFLYSKLTVDKSRWQQGNVFSCSVMHEALHNHYTQKSLSLSPGK

SEQ ID NO: 10 - protein, 121 aa, Murine
  mAb-001 VH
QVHLQQSGAELAKPGASVKLSCKASGYTFNDYWMHWVKERPGQGLEWIGYINPSSGFTKYHQNFKDKATLTADKSSSTAYMQLSSLTYDDSAVYYCARQYDYDEDWYFDVWGTGTTVTVSS

SEQ ID NO: 11 - protein, 112 aa, Murine
  mAb-001VL
DIVMSQSPSSLAVSAGEKVTMSCKSSQSLLNSRTRKNFLAWYQQKPGQSPKLLIYWASTRESGVPDRFTGRGSGTDFTLTISSVQAEDLAVYYCKQSFNLFTFGSGTKLEIK

SEQ ID NO: 12 - protein, 5 aa, Murine
  mAb-001 HCDR1
DYWMH

SEQ ID NO: 13 - protein, 17 aa, Murine
  mAb-001 HCDR2
YINPSSGFTKYHQNFKD

SEQ ID NO: 14 - protein, 12 aa, Murine
  mAb-001 HCDR3
QYDYDEDWYFDV

SEQ ID NO: 15 - protein, 17 aa, Murine
  mAb-001 LCDR1
KSSQSLLNSRTRKNFLA

SEQ ID NO: 16 - protein, 7 aa, Murine
  mAb-001 LCDR2
WASTRES

SEQ ID NO: 17 - protein, 8 aa, Murine
  mAb-001 LCDR3
KQSFNLFT

SEQ ID NO: 18 - protein, 121 aa, ARTIFICIAL
  h001-VH.1
QVQLVQSGAEVKKPGASVKVSCKASGYTFTDYWMHWVRQAPGQGLEWMGYINPSSGFTKYHQNFKDRVTMTRDTSISTAYMELSRLRSDDTAVYYCARQYDYDEDWYFDVWGQGTTVTVSS

SEQ ID NO: 19 - protein, 121 aa, ARTIFICIAL
  h001-VH.1A
QVQLVQSGAEVKKPGASVKVSCKASGYTFNDYWMHWVRQAPGQGLEWMGYINPSSGFTKYHQNFKDRVTMTRDTSISTAYMELSRLRSDDTAVYYCARQYDYDEDWYFDVWGQGTTVTVSS

SEQ ID NO: 20 - protein, 121 aa, ARTIFICIAL
  h001-VH.1B
QVQLVQSGAEVKKPGASVKVSCKASGYTFTDYWMHWVRQAPGQGLEWMGYINPSSGFTKYHQNFKDRVTMTRDTSISTAYMELSRLTSDDTAVYYCARQYDYDEDWYFDVWGQGTTVTVSS

SEQ ID NO: 21 - protein, 121 aa, ARTIFICIAL
  h001-VH.1C
QVQLVQSGAEVKKPGASVKVSCKASGYTFNDYWMHWVRQAPGQGLEWMGYINPSSGFTKYHQNFKDRVTMTRDTSISTAYMELSRLTSDDTAVYYCARQYDYDEDWYFDVWGQGTTVTVSS

SEQ ID NO: 22 - protein, 121 aa, ARTIFICIAL
  h001-VH.1D
QVQLVQSGAEVKKPGASVKVSCKASGYTFNDYWMHWVRQAPGQGLEWMGYINPSSGFTKYHQNFKDRVTMTADKSISTAYMELSRLTSDDTAVYYCARQYDYDEDWYFDVWGQGTTVTVSS

SEQ ID NO: 23 - protein, 121 aa, ARTIFICIAL
  h001-VH.1E
QVQLVQSGAEVKKPGASVKVSCKASGYTFNDYWMHWVKQAPGQGLEWIGYINPSSGFTKYHQNFKDKATLTADKSISTAYMELSRLTSDDTAVYYCARQYDYDEDWYFDVWGQGTTVTVSS

SEQ ID NO: 24 - protein, 112 aa, ARTIFICIAL
  h001-VL.1 (CDR grafting)
DIQMTQSPSSLSASVGDRVTITCKSSQSLLNSRTRKNFLAWYQQKPGKAPKLLIYWASTRESGVPSRFSGSGSGTDFTLTISSLQPEDFATYYCKQSFNLFTFGQGTKLEIK

SEQ ID NO: 25 - protein, 112 aa, ARTIFICIAL
  h001-VL.1A
DIQMTQSPSSLSASVGDRVTITCKSSQSLLNSRTRKNFLAWYQQKPGKAPKLLIYWASTRESGVPDRFSGSGSGTDFTLTISSLQPEDFATYYCKQSFNLFTFGQGTKLEIK

SEQ ID NO: 26 - protein, 112 aa, ARTIFICIAL
  h001-VL.1B
DIQMSQSPSSLSASVGDRVTITCKSSQSLLNSRTRKNFLAWYQQKPGKAPKLLIYWASTRESGVPDRFSGSGSGTDFTLTISSLQPEDFATYYCKQSFNLFTFGQGTKLEIK

SEQ ID NO: 27 - protein, 112 aa, ARTIFICIAL
  h001-VL.1C
DIVMSQSPSSLSASVGDRVTITCKSSQSLLNSRTRKNFLAWYQQKPGKSPKLLIYWASTRESGVPDRFSGSGSGTDFTLTISSLQPEDFATYYCKQSFNLFTFGQGTKLEIK

SEQ ID NO: 28 - protein, 451 aa, ARTIFICIAL
  h001-4-IgG1 Heavy chain amino acid sequence
QVQLVQSGAEVKKPGASVKVSCKASGYTFTDYWMHWVRQAPGQGLEWMGYINPSSGFTKYHQNFKDRVTMTRDTSISTAYMELSRLRSDDTAVYYCARQYDYDEDWYFDVWGQGTTVTVSSASTKGPSVFPLAPSSKSTSGGTAALGCLVKDYFPEPVTVSWNSGALTSGVHTFPAVLQSSGLYSLSSVVTVPSSSLGTQTYICNVNHKPSNTKVDKKVEPKSCDKTHTCPPCPAPELLGGPSVFLFPPKPKDTLMISRTPEVTCVVVDVSHEDPEVKFNWYVDGVEVHNAKTKPREEQYNSTYRVVSVLTVLHQDWLNGKEYKCKVSNKALPAPIEKTISKAKGQPREPQVYTLPPSRDELTKNQVSLTCLVKGFYPSDIAVEWESNGQPENNYKTTPPVLDSDGSFFLYSKLTVDKSRWQQGNVFSCSVMHEALHNHYTQKSLSLSPGK

SEQ ID NO: 29 - DNA, 1413 bp, ARTIFICIAL
  h001-4-IgG1 Heavy chain DNA sequence
atggagtttgggctgagctggctttttcttgtcgcgattcttaagggtgtccagtgccaggtgcagctggtgcagagcggcgctgaggtgaagaagcccggagcgagcgtaaaggtgagctgcaaggccagcggatacaccttcaccgactactggatgcactgggtgaggcaggccccaggacagggcctggagtggatgggctacatcaaccccagcagcggctttaccaagtatcaccagaacttcaaagacagggtgaccatgaccagggacaccagcatcagcaccgcctacatggagctgagcaggctgaggagcgacgacaccgccgtgtactactgcgccaggcaatacgactacgacgaggactggtacttcgacgtgtggggccaaggaaccaccgtgactgtgagcagcgcttcgaccaagggcccatcggtcttccccctggcaccctcctccaagagcacctctgggggcacagcggccctgggctgcctggtcaaggactacttccccgaaccggtgacggtgtcgtggaactcaggcgccctgaccagcggcgtgcacaccttcccggctgtcctacagtcctcaggactctactccctcagcagcgtggtgaccgtgccctccagcagcttgggcacccagacctacatctgcaacgtgaatcacaagcccagcaacaccaaggtggacaagaaagttgagcccaaatcttgtgacaaaactcacacatgcccaccgtgcccagcacctgaactcctggggggaccgtcagtcttcctcttccccccaaaacccaaggacaccctcatgatctcccggacccctgaggtcacatgcgtggtggtggacgtgagccacgaagaccctgaggtcaagttcaactggtacgtggacggcgtggaggtgcataatgccaagacaaagccgcgggaggagcagtacaacagcacgtaccgtgtggtcagcgtcctcaccgtcctgcaccaggactggctgaatggcaaggagtacaagtgcaaggtctccaacaaagccctcccagcccccatcgagaaaaccatctccaaagccaaagggcagccccgagaaccacaggtgtacaccctgcccccatcccgggatgagctgaccaagaaccaggtcagcctgacctgcctggtcaaaggcttctatcccagcgacatcgccgtggagtgggagagcaatgggcagccggagaacaactacaagaccacgcctcccgtgctggactccgacggctccttcttcctctacagcaagctcaccgtggacaagagcaggtggcagcaggggaacgtcttctcatgctccgtgatgcatgaggctctgcacaaccactacacgcagaagagcctctccctgtctccgggtaaatga

SEQ ID NO: 30 - protein, 219 aa, ARTIFICIAL
  h001-4-kappa Light chain amino acid sequence
DIVMSQSPSSLSASVGDRVTITCKSSQSLLNSRTRKNFLAWYQQKPGKSPKLLIYWASTRESGVPDRFSGSGSGTDFTLTISSLQPEDFATYYCKQSFNLFTFGQGTKLEIKRTVAAPSVFIFPPSDEQLKSGTASVVCLLNNFYPREAKVQWKVDNALQSGNSQESVTEQDSKDSTYSLSSTLTLSKADYEKHKVYACEVTHQGLSSPVTKSFNRGEC

SEQ ID NO: 31 - DNA, 726 bp, ARTIFICIAL
  h001-4-kappa Light chain DNA sequence
atggacatgcgcgtgcccgcccagctgctgggcctgctgctgctgtggttccccggctcgcgatgcgacatcgtgatgtctcagagcccatctagcctgagcgccagcgtgggcgacagggtaaccatcacctgcaagagcagccaaagcctgctgaacagcaggacccgcaagaacttcctggcttggtatcagcagaagcccggcaagtctcccaagttgctgatctactgggccagcaccagggagagcggcgtgcccgacaggttcagcggctccggcagcggcaccgacttcaccctgaccatctctagtctgcagcccgaggacttcgccacctactactgcaagcagagcttcaatctgttcaccttcggccagggcaccaagctggagatcaagcgtacggtggctgcaccatctgtcttcatcttcccgccatctgatgagcagttgaaatctggaactgcctctgttgtgtgcctgctgaataacttctatcccagagaggccaaagtacagtggaaggtggataacgccctccaatcgggtaactcccaggagagtgtcacagagcaggacagcaaggacagcacctacagcctcagcagcaccctgacgctgagcaaagcagactacgagaaacacaaagtctacgcctgcgaagtcacccatcagggcctgagctcgcccgtcacaaagagcttcaacaggggagagtgttga

SEQ ID NO: 32 - protein, 451 aa, ARTIFICIAL
  h001-4-IgG1-YTE Heavy chain amino acid sequence
QVQLVQSGAEVKKPGASVKVSCKASGYTFTDYWMHWVRQAPGQGLEWMGYINPSSGFTKYHQNFKDRVTMTRDTSISTAYMELSRLRSDDTAVYYCARQYDYDEDWYFDVWGQGTTVTVSSASTKGPSVFPLAPSSKSTSGGTAALGCLVKDYFPEPVTVSWNSGALTSGVHTFPAVLQSSGLYSLSSVVTVPSSSLGTQTYICNVNHKPSNTKVDKKVEPKSCDKTHTCPPCPAPELLGGPSVFLFPPKPKDTLYITREPEVTCVVVDVSHEDPEVKFNWYVDGVEVHNAKTKPREEQYNSTYRVVSVLTVLHQDWLNGKEYKCKVSNKALPAPIEKTISKAKGQPREPQVYTLPPSRDELTKNQVSLTCLVKGFYPSDIAVEWESNGQPENNYKTTPPVLDSDGSFFLYSKLTVDKSRWQQGNVFSCSVMHEALHNHYTQKSLSLSPGK

SEQ ID NO: 33 - DNA, 1413 bp, ARTIFICIAL
  h001-4-IgG1-YTE Heavy chain DNA sequence
atggagtttgggctgagctggctttttcttgtcgcgattcttaagggtgtccagtgccaggtgcagctggtgcagagcggcgctgaggtgaagaagcccggagcgagcgtaaaggtgagctgcaaggccagcggatacaccttcaccgactactggatgcactgggtgaggcaggccccaggacagggcctggagtggatgggctacatcaaccccagcagcggctttaccaagtatcaccagaacttcaaagacagggtgaccatgaccagggacaccagcatcagcaccgcctacatggagctgagcaggctgaggagcgacgacaccgccgtgtactactgcgccaggcaatacgactacgacgaggactggtacttcgacgtgtggggccaaggaaccaccgtgactgtgagcagcgcttcgaccaagggcccatcggtcttccccctggcaccctcctccaagagcacctctgggggcacagcggccctgggctgcctggtcaaggactacttccccgaaccggtgacggtgtcgtggaactcaggcgccctgaccagcggcgtgcacaccttcccggctgtcctacagtcctcaggactctactccctcagcagcgtggtgaccgtgccctccagcagcttgggcacccagacctacatctgcaacgtgaatcacaagcccagcaacaccaaggtggacaagaaagttgagcccaaatcttgtgacaaaactcacacatgcccaccgtgcccagcacctgaactcctggggggaccgtcagtcttcctcttccccccaaaacccaaggacaccctctacatcacccgggagcctgaggtcacatgcgtggtggtggacgtgagccacgaagaccctgaggtcaagttcaactggtacgtggacggcgtggaggtgcataatgccaagacaaagccgcgggaggagcagtacaacagcacgtaccgtgtggtcagcgtcctcaccgtcctgcaccaggactggctgaatggcaaggagtacaagtgcaaggtctccaacaaagccctcccagcccccatcgagaaaaccatctccaaagccaaagggcagccccgagaaccacaggtgtacaccctgcccccatcccgggatgagctgaccaagaaccaggtcagcctgacctgcctggtcaaaggcttctatcccagcgacatcgccgtggagtgggagagcaatgggcagccggagaacaactacaagaccacgcctcccgtgctggactccgacggctccttcttcctctacagcaagctcaccgtggacaagagcaggtggcagcaggggaacgtcttctcatgctccgtgatgcatgaggctctgcacaaccactacacgcagaagagcctctccctgtctccgggtaaatga